European Patent Specification EP 4 153 769 B1, published March 26, 2025. Title: DISPOSITIF DE DETECTION D'UNE BACTERIE D'INTERET. Applicant: VETOPHAGE NEOVIA. The sequence listing filed with the application follows.

SEQUENCE LISTING (6 sequences)

SEQ ID NO: 1 - protein, 458 aa, Staphylococcus aureus
MALNFTTITENNVIRDLTTQVNNIGEELTKERNIFDITDDLVYNFNKSQKIKLTDDKGLTKSYGNITALRDIKEPGYYYIGARTLATLLDRPDMESLDVVLHVVPLDTSSKVVQHLYTLSTNNNQIKMLYRFVSGNSSSEWQFIQGLPSNKNAVISGTNILDIASPGVYFVMGMTGGMPSGVSSGFLDLSVDANDNRLARLTDAETGKEYTSIKKPTGTYTAWKKEFEPKDMEKYLLSSIRDDGSASFPLLVYTSDSKTFQQAIIDHIDRTGQTTFTFYVQGGVSGSPMSNSCRGLFMSDTPNTSSLHGVYNAIGTDGRNVTGSVVGSNWTSPKTSPSHKELWTGAQSFLSTGTTKNLSDDISNYSYVEVYTTHKTTEKTKGNDNTGTICHKFYLDGSGTYVCSGTFVSGDRTDTKPPITEFYRVGVSFKGSTWTLVDSAVQNSKTQYVTRIIGINMP

SEQ ID NO: 2 - protein, 636 aa, Staphylococcus aureus
MENLYLIKDLGALAGRDYRAKEIQNLQRIEQFALGLTTEFKLHQKAKTMQHFAEQIYYNGRSQAAVNKSLQSQINALVVAPRNNSANEIVQARVNVNGETFDTLKEHLDDWETKTQINKEETIRELNKTKQEILDIEYRFEPDKQEFLFVTELAPLTNAVMQSFWFDNRTGIVYMTQARNNGYMLSRLRPNGQFIDSSLIVGGGHGTHNGYRYIDDELWIYSFILNGNNENTLVRFKYTPNVEISYGKYGMQDVFTGHPEKPYITPVINEKENKILYRIERPRSQWELENSMNYIEIRSLDDVDKNIDKVLHKISIPMRLTNETQPMQGVTFDEKYLYWYTGDSNPNNRNYLTAFDLETGEEAYQVNADYGGTLDSFPGEFAEAEGLQIYYDKDSGKKALMLGVTVGGDGNRTHRIFMIGQRGILEILHSRGVPFIMSDTGGRVKPLPMRPDKLKNLGMLTEPGLYYLYTDHTVQIDDFPLPREWRDAGWFLEVKPPQTGGDVIQILTRNSYARNMMTFERVLSGRTGDISDWNYVPKNSGKWERVPSFITKMSDINIVGMSFYLTTDDTKRFTDFPTERKGVAGWNLYVEASNTGGFVHRLVRNSVTASAEILLKNYDSKTSSGPWTLHEGRIIS

SEQ ID NO: 3 - protein, 467 aa, Staphylococcus aureus
MALNFTTITENNVIRDLTTQVNNIGEELTKDRNVFDITDDLVYSFNKSQKIKLTDDKGLAKIHSTTSVLRDIKKPGYYYISARTLATMVDKPDMESIDVVLHVLPVDTTNRIVQQLYTLSVNNNQIKTLYRFVSGSSSSEWQFIQGLPNNKNMVISGANPLEMTTPGVYFVTGMIEGMPDNVSAGFLELSVDSNDNRLAKVTDIETGKHYTNIKKASGVYTGWKKELEPEDLQQYLPSRVNPSEGEASYNISIYKSDDLSFPKAIENHIIETRETFITFYCQGGVAENPGGLASIRGIVMIDNPEDYKRNGFYGSYIALTTSGVVISGAISGGTWYPPKTSPTYKELWTGAQAFSSTGISKKLADDISNYSYVEIYIKYKTVEKTKGSDDAGTICHKFYLDGSNICVCSGTFVSGDRTATKPPITEFYRLGIKFKGSTWTIDEGAIQSPKTQYVTRITNFGCLYKVV

SEQ ID NO: 4 - protein, 632 aa, Staphylococcus aureus
MAYGLITSLHSITGEKVVAQHEYNYRLLDNGMSKLEKMFIYHQKEEIYAHTANQIKYLNGSVSDFLAYLNGRFSNMVLGHNGDGINEVKDARVDNTGYAHPTLQDRLYHDYSTLDAFTKKVEKVVGEHYKEYQATEYRFEPKEQEPEFITDLSPYTNAVMQSFWVDPRTKIIYMTQARPGNHYMLSRLKPNGQFIDRLLVKNGGHGTHNAYRYIGNELWIYSAVLDANNNNKFVRFKYRSGEMTYGNEMQDVMPNVFNDRYTSAIYNPIENLMIFRREYKTSEQQAKNSLNFIEVRSVDDIDKGIDKVLYQMDIPMEYSSLTQPMQGIAYDAGVLYWYTGDSNPANPNYLQGFDIKTKELLFKRRIDIGGVNNNFKGDFQEAEGLDMYYDLETGRKALLIGVTIGPGNNRHHSIYSIGQRGVNQFLKNIAPQVSMTDSGGRVKPLPVQNPAYLSDVTEVGNYYLYSQDTQNALDFPLPKEFRDAGWFFDVLPGHYNGALRQVLTRNSTGRNMLKFERVIDIFNKKNNGSWNFNPQSAGFWEHIPKSITKLSDLKIVGLDFYITTEESKRFTDFPKDFKGIAGWILEVKSNTPGNTTQVLRRNNFPSAHQFLLRNFGTGGVGKWSLFEGKVVE

SEQ ID NO: 5 - protein, 636 aa, Staphylococcus aureus
MENLYLIKDLGALAGRDYRAKEIQNLQRIEQFALGLTTEFKLHQKAKTIQHFAEQIYYNGRSQAAVNKSLQSQINALVVAPRNNSANEIVQARVNVNGETFDTLKEHLDDWETKTQNNKEETIRELNKTKQEILDIEYRFEPDKQEFLFVTELAPLTNAVMQSFWFDNRTGIVYMTQARNNGYMLSRLRPNGQFIDSSLIVGGGHGTHNGYRYIDDELWIYSFILNGNNENTLVRFKYTPNVEISYGKYDMQDVFTGHPEKPYITPVINEKENKILYRIERPRSQWELENSMNYIEIRSLDDVDKNIDKVLHKISIPMRLTNENQPMQGVTFDEKYLYWYTGDSNPNNRNYLTAFDLETGEEAYQVNADYGGTLDSFPGEFAEAEGLQIYYDKDSGKKALMLGVTVGGDGNRTHRIFMIGQRGILEILHSRGVPFIMSDTGGRVKPLPMRPDKLKNLGMLTEPGLYYLYTDHTVQIDDFPLPREWRDAGWFLEVKPPQTGGDVIQILTRNSYARNMMTFERVLSGRTGDISDWNYVPKNSGKWERVPSFITKMSDINIVGMSFYLTTDDTKRFTDFPTERKGVAGWNLYVEASNTGGFVHRLVRNSVTASAEILLKNYDSKTSSGPWTLHEGRIIS

SEQ ID NO: 6 - protein, 636 aa, Staphylococcus aureus
MENLYLIKDLGALAGRDYRAKEIQNLQRIEQFALGLTTEFKLHQKAKTIQHFAEQIYYNGRSQAAVNKSLQSQINALVLAPRNNSANEIVQARVNVNGETFDTLKEHLDDWETKTQNNKEETIRELNKAKQQILDIEYRFEPDKQEFLFVTELAPLTNAVMQSFWFDNRTGIVYMTQARNNGYMLSRLRPNGQFIDSSLIVGGGHGTHNGYRYIDDELWIYSFILNGNNENTLVRFKYTPNVEISYGKYGMQDVFTGHPEKPYITPVINEKENKILYRIERPRSQWELENSMNYIEIRSLDDVDKNIDKVLYKISIPMRLTNETQPMQGVTFDEKYLYWYTGDSNPNNRNYLTAFDLETGEEAYQVNADYGGTLDSFPGEFAEAEGLQIYYDKDSGKKALMLGVTVGGDGNRTHRIFMIGQRGILEILHSRGVPFIMSDTGGRVKPLPMRPDKLTNLGMLTEPGLYYLYTDHTVQIDDFPLPREWRDAGWFLEVKPPQTGGDVIQILTRNSYARNMMTFERVLSGRTGDISDWNYVPKNSGKWERVPSFITKMSDINIVGMSFYLTTDDTKRFTDFPTERKGVAGWNLYVEASNTGGFVHRLVRNSVTASCEILLKNYDSKTSSGPWTLHEGRIIS